European Patent Application EP 4 703 376 A1, published March 4, 2026. Title: RECOMBINANT SMALL-MOLECULE COLLAGEN, EXPRESSION SYSTEM THEREOF, AND PREPARATION METHOD THEREOF. Applicant: JIANGSU TRAUTEC MEDICAL TECHNOLOGY CO., LTD. The sequence listing filed with the application follows.

SEQUENCE LISTING (81 sequences)

SEQ ID NO: 1 - protein, 96 aa, Homo sapiens
  source 1..96: note = Recombinant small-molecule collagen 3A5D1NT
DGNPGSDGLPGRDGSPGGKGDRGENGSPGAPGAPGHPGPPGPVGPAGKSGDRGESGPAGPAGAPGPAGSRGAPGPQGPRGDKGETGERGAAGIKGH

SEQ ID NO: 2 - protein, 101 aa, synthetic construct
  source 1..101: note = Recombinant small-molecule collagen 3A5D1
DGNPGSDGLPGRDGSPGGKGDRGENGSPGAPGAPGHPGPPGPVGPAGKSGDRGESGPAGPAGAPGPAGSRGAPGPQGPRGDKGETGERGAAGIKGHHHHHH

SEQ ID NO: 3 - protein, 50 aa, Homo sapiens
  source 1..50: note = Recombinant small-molecule collagen 3A5D2NT
GKSGDRGESGPAGPAGAPGPAGSRGAPGPQGPRGDKGETGERGAAGIKGH

SEQ ID NO: 4 - protein, 55 aa, synthetic construct
  source 1..55: note = Recombinant small-molecule collagen 3A5D2
GKSGDRGESGPAGPAGAPGPAGSRGAPGPQGPRGDKGETGERGAAGIKGHHHHHH

SEQ ID NO: 5 - protein, 82 aa, Homo sapiens
  source 1..82: note = Recombinant small-molecule collagen 17S1NNT
GPPGSGEKGERGAAGEPGPHGPPGVPGSVGPKGSSGSPGPQGPPGPVGLQGLRGEVGLPGVKGDKGPMGPPGPKGDQGEKGP

SEQ ID NO: 6 - protein, 88 aa, synthetic construct
  source 1..88: note = Recombinant small-molecule collagen 17S1N
GPPGSGEKGERGAAGEPGPHGPPGVPGSVGPKGSSGSPGPQGPPGPVGLQGLRGEVGLPGVKGDKGPMGPPGPKGDQGEKGPHHHHHH

SEQ ID NO: 7 - protein, 59 aa, Homo sapiens
  source 1..59: note = Recombinant small-molecule collagen 17S3NT
GVPGSVGPKGSSGSPGPQGPPGPVGLQGLRGEVGLPGVKGDKGPMGPPGPKGDQGEKGP

SEQ ID NO: 8 - protein, 65 aa, synthetic construct
  source 1..65: note = Recombinant small-molecule collagen 17S3
GVPGSVGPKGSSGSPGPQGPPGPVGLQGLRGEVGLPGVKGDKGPMGPPGPKGDQGEKGPHHHHHH

SEQ ID NO: 9 - DNA, 291 bp, synthetic construct
  source 1..291: mol_type = other DNA; note = Codon-optimized DNA sequence encoding recombinant small-molecule collagen 3A5D1NT
gacgggaacccagggagtgatggcctgccaggacgcgatggctccccgggagggaagggggaccggggcgaaaatggttcgcccggagcgccgggtgctcctggtcaccctggtccgcccgggcctgtcggaccagccggcaaatctggcgatcgaggagagagcggcccagctggtcccgctggggcaccaggtccggctgggtcaaggggtgcacctggccctcagggacccagaggagacaagggcgagaccggtgaacgtggagccgcgggtattaaaggtcactaa

SEQ ID NO: 10 - DNA, 306 bp, synthetic construct
  source 1..306: mol_type = other DNA; note = Codon-optimized DNA sequence encoding recombinant small-molecule collagen 3A5D1
gacgggaacccagggagtgatggcctgccaggacgcgatggctccccgggagggaagggggaccggggcgaaaatggttcgcccggagcgccgggtgctcctggtcaccctggtccgcccgggcctgtcggaccagccggcaaatctggcgatcgaggagagagcggcccagctggtcccgctggggcaccaggtccggctgggtcaaggggtgcacctggccctcagggacccagaggagacaagggcgagaccggtgaacgtggagccgcgggtattaaaggtcaccatcatcatcaccactaa

SEQ ID NO: 11 - DNA, 159 bp, synthetic construct
  source 1..159: mol_type = other DNA; note = Codon-optimized DNA sequence encoding recombinant small-molecule collagen 3A5D2NT
gaggcagggaagtccggtgacaggggggagagcggacctgctggtcctgctggagccccgggtcctgctggctctcgcggcgcgccaggaccgcaaggcccacgtggtgataaaggagaaacaggggaaagaggggccgcaggtattaaaggtcactaa

SEQ ID NO: 12 - DNA, 174 bp, synthetic construct
  source 1..174: mol_type = other DNA; note = Codon-optimized DNA sequence encoding recombinant small-molecule collagen 3A5D2
gaggcagggaagtccggtgacaggggggagagcggacctgctggtcctgctggagccccgggtcctgctggctctcgcggcgcgccaggaccgcaaggcccacgtggtgataaaggagaaacaggggaaagaggggccgcaggtattaaaggtcaccatcaccatcatcactaa

SEQ ID NO: 13 - DNA, 255 bp, synthetic construct
  source 1..255: mol_type = other DNA; note = Codon-optimized DNA sequence encoding recombinant small-molecule collagen 17S1NNT
gaggccggccctccaggttcgggcgagaaaggggaaagaggggcggcaggagaacccggaccccacggtcctcctggagtcccgggttccgtaggcccaaaaggcagctctggaagtccggggccacaagggcctccaggccccgttggtttacagggtctacgcggcgaagtgggattgccaggggtaaagggcgacaagggtccgatgggacctcccggtcctaagggtgatcaaggggagaaaggaccgtaa

SEQ ID NO: 14 - DNA, 273 bp, synthetic construct
  source 1..273: mol_type = other DNA; note = Codon-optimized DNA sequence encoding recombinant small-molecule collagen 17S1N
gaggccggccctccaggttcgggcgagaaaggggaaagaggggcggcaggagaacccggaccccacggtcctcctggagtcccgggttccgtaggcccaaaaggcagctctggaagtccggggccacaagggcctccaggccccgttggtttacagggtctacgcggcgaagtgggattgccaggggtaaagggcgacaagggtccgatgggacctcccggtcctaagggtgatcaaggggagaaaggaccgcatcaccaccatcatcattaa

SEQ ID NO: 15 - DNA, 186 bp, synthetic construct
  source 1..186: mol_type = other DNA; note = Codon-optimized DNA sequence encoding recombinant small-molecule collagen 17S3NT
gaagccggtgtccctggctctgttggaccgaagggtagttcgggaagcccagggcctcaggggccgcccggacccgtaggtctgcaggggctcagaggagaggtgggcctacctggcgtcaagggcgacaaaggtccaatggggccgcctggaccaaaaggggatcaaggtgaaaaaggcccctaa

SEQ ID NO: 16 - DNA, 204 bp, synthetic construct
  source 1..204: mol_type = other DNA; note = Codon-optimized DNA sequence encoding recombinant small-molecule collagen 17S3
gaagccggtgtccctggctctgttggaccgaagggtagttcgggaagcccagggcctcaggggccgcccggacccgtaggtctgcaggggctcagaggagaggtgggcctacctggcgtcaagggcgacaaaggtccaatggggccgcctggaccaaaaggggatcaaggtgaaaaaggcccccaccatcatcaccatcactaa

SEQ ID NO: 17 - protein, 307 aa, Homo sapiens
  source 1..307: note = Mature peptide sequence of human carboxypeptidase B
ATGHSYEKYNKWETIEAWTQQVATENPALISRSVIGTTFEGRAIYLLKVGKAGQNKPAIFMDCGFHAREWISPAFCQWFVREAVRTYGREIQVTELLDKLDFYVLPVLNIDGYIYTWTKSRFWRKTRSTHTGSSCIGTDPNRNFDAGWCEIGASRNPCDETYCGPAAESEKETKALADFIRNKLSSIKAYLTIHSYSQMMIYPYSYAYKLGENNAELNALAKATVKELASLHGTKYTYGPGATTIYPAAGGSDDWAYDQGIRYSFTFELRDTGRYGFLLPESQIRATCEETFLAIKYVASYVLEHLY

SEQ ID NO: 18 - protein, 307 aa, Rattus norvegicus
  source 1..307: note = Mature peptide sequence of rat carboxypeptidase B
ASGHSYTKYNKWETIEAWIQQVATDNPDLVTQSVIGTTFEGRNMYVLKIGKTRPNKPAIFIDCGFHAREWISPAFCQWFVREAVRTYNQEIHMKQLLDELDFYVLPVVNIDGYVYTWTKDRMWRKTRSTMAGSSCLGVRPNRNFNAGWCEVGASRSPCSETYCGPAPESEKETKALADFIRNNLSTIKAYLTIHSYSQMMLYPYSYDYKLPENYEELNALVKGAAKELATLHGTKYTYGPGATTIYPAAGGSDDWSYDQGIKYSFTFELRDTGFFGFLLPESQIRQTCEETMLAVKYIANYVREHLY

SEQ ID NO: 19 - protein, 136 aa, Saccharomyces cerevisiae
  source 1..136: note = Amino acid sequence at positions 679-814 in full-length amino acid sequence of Kex2
YFLTIFLIGATFLVLYFMFFMKSRRRIRRSRAETYEFDIIDTDSEYDSTLDNGTSGITEPEEVEDFDFDLSDEDHLASLSSSENGDAEHTIDSVLTNENPFSDPIKQKFPNDANAESASNKLQELQPDVPPSSGRS

SEQ ID NO: 20 - protein, 97 aa, Komagataella phaffii
  source 1..97: note = Amino acid sequence at positions 681-777 in full-length amino acid sequence of Kex2
YLAFLLGLGFLICIIFLFTNRNKLERRQRRNRRDEYEFDLIPADDDFDTEEDQEANSQFTLDSDAELMFEDTSQREASPHEYQDSLGSNEHPKRAAL

SEQ ID NO: 21 - protein, 10 aa, synthetic construct
  source 1..10: note = Linker
GGSGSGSGGS

SEQ ID NO: 22 - protein, 414 aa, synthetic construct
  source 1..414: note = CPB positioning fusion functional protein HCPB-PPKEX2
ATGHSYEKYNKWETIEAWTQQVATENPALISRSVIGTTFEGRAIYLLKVGKAGQNKPAIFMDCGFHAREWISPAFCQWFVREAVRTYGREIQVTELLDKLDFYVLPVLNIDGYIYTWTKSRFWRKTRSTHTGSSCIGTDPNRNFDAGWCEIGASRNPCDETYCGPAAESEKETKALADFIRNKLSSIKAYLTIHSYSQMMIYPYSYAYKLGENNAELNALAKATVKELASLHGTKYTYGPGATTIYPAAGGSDDWAYDQGIRYSFTFELRDTGRYGFLLPESQIRATCEETFLAIKYVASYVLEHLYGGSGSGSGGSYLAFLLGLGFLICIIFLFTNRNKLERRQRRNRRDEYEFDLIPADDDFDTEEDQEANSQFTLDSDAELMFEDTSQREASPHEYQDSLGSNEHPKRAAL

SEQ ID NO: 23 - DNA, 1245 bp, synthetic construct
  source 1..1245: mol_type = other DNA; note = DNA sequence encoding HCPB-PPKEX2
gcgacaggacacagctatgagaaatacaacaaatgggagacaatagaggcgtggacgcagcaggtggccaccgaaaacccggctcttatatctcgttctgtcatcggaaccactttcgaaggccgagccatctacctacttaaggtcggcaaagcaggtcaaaacaaaccagcaatctttatggactgtggattccatgctagggagtggatctcaccagcattctgtcagtggttcgtacgggaggcggttcgaacgtatggtagagaaattcaggtcacagagctgttggacaagctcgatttttatgtactacctgtgctgaacattgatgggtatatttatacctggactaagtcccgcttttggcgcaagacgcggagtacgcacactgggtcctcttgcatcggaacagaccccaaccgtaatttcgatgcaggctggtgcgagataggggctagtcgtaatccgtgcgacgagacgtactgcgggcccgcggctgaatcagaaaaggaaactaaggcgcttgcggatttcattagaaataaactttccagtatcaaagcgtatttgaccatacactcgtatagccaaatgatgatctacccctactcctacgcgtataaacttggtgaaaacaacgccgaactgaatgccctcgccaaggcaactgtgaaggagctagcaagcttgcatggaactaaatacacttacgggcctggtgccacaaccatatacccggctgccgggggtagtgacgattgggcttatgatcagggtataaggtatagctttacgttcgagctgcgtgatacgggccgttatggattcttgctccctgagtctcaaattagggctacctgtgaagaaacatttctggctattaaatatgttgcatcttacgtattagaacatttatacggaggctcgggatctgggtcgggtggctcatacctagccttcttactgggcctcggttttttaatatgtattatcttcctctttacaaaccggaataagttggaacgccggcaaaggcgaaatcgccgagatgaatatgaatttgaccttattcccgcagatgacgactttgatactgaggaagatcaagaagcgaattcacaatttaccttagactcagacgccgagctaatgtttgaagatacctcgcaacgagaggcgtccccacatgagtaccaggactcgttgggcagcaatgagcacccaaaaagagctgcattataa

SEQ ID NO: 24 - protein, 453 aa, synthetic construct
  source 1..453: note = CPB positioning fusion functional protein HCPB-SCKEX2
ATGHSYEKYNKWETIEAWTQQVATENPALISRSVIGTTFEGRAIYLLKVGKAGQNKPAIFMDCGFHAREWISPAFCQWFVREAVRTYGREIQVTELLDKLDFYVLPVLNIDGYIYTWTKSRFWRKTRSTHTGSSCIGTDPNRNFDAGWCEIGASRNPCDETYCGPAAESEKETKALADFIRNKLSSIKAYLTIHSYSQMMIYPYSYAYKLGENNAELNALAKATVKELASLHGTKYTYGPGATTIYPAAGGSDDWAYDQGIRYSFTFELRDTGRYGFLLPESQIRATCEETFLAIKYVASYVLEHLYGGSGSGSGGSYFLTIFLIGATFLVLYFMFFMKSRRRIRRSRAETYEFDIIDTDSEYDSTLDNGTSGITEPEEVEDFDFDLSDEDHLASLSSSENGDAEHTIDSVLTNENPFSDPIKQKFPNDANAESASNKLQELQPDVPPSSGRS

SEQ ID NO: 25 - DNA, 1362 bp, synthetic construct
  source 1..1362: mol_type = other DNA; note = DNA sequence encoding HCPB-SCKEX2
gcgacaggacacagctatgagaaatacaacaaatgggagacaatagaggcgtggacgcagcaggtggccaccgaaaacccggctcttatatctcgttctgtcatcggaaccactttcgaaggccgagccatctacctacttaaggtcggcaaagcaggtcaaaacaaaccagcaatctttatggactgtggattccatgctagggagtggatctcaccagcattctgtcagtggttcgtacgggaggcggttcgaacgtatggtagagaaattcaggtcacagagctgttggacaagctcgatttttatgtactacctgtgctgaacattgatgggtatatttatacctggactaagtcccgcttttggcgcaagacgcggagtacgcacactgggtcctcttgcatcggaacagaccccaaccgtaatttcgatgcaggctggtgcgagataggggctagtcgtaatccgtgcgacgagacgtactgcgggcccgcggctgaatcagaaaaggaaactaaggcgcttgcggatttcattagaaataaactttccagtatcaaagcgtatttgaccatacactcgtatagccaaatgatgatctacccctactcctacgcgtataaacttggtgaaaacaacgccgaactgaatgccctcgccaaggcaactgtgaaggagctagcaagcttgcatggaactaaatacacttacgggcctggtgccacaaccatatacccggctgccgggggtagtgacgattgggcttatgatcagggtataaggtatagctttacgttcgagctgcgtgatacgggccgttatggattcttgctccctgagtctcaaattagggctacctgtgaagaaacatttctggctattaaatatgttgcatcttacgtattagaacatttatacggaggctcgggatctgggtcgggtggctcatatttcctcacaatattcttaataggcgcaacgtttttagtgctgtattttatgtttttcatgaaatcaaggcggagaatccggcgttcacgcgcggagacctacgagttcgacatcatagatactgactcggaatacgattcaaccctggataacgggacctcgggtattactgaacccgaggaggtagaggatttcgatttcgacctctctgacgaagatcatctagccagtctatcgtccagtgaaaatggagatgctgaacacacaatcgacagcgtccttacgaatgagaacccgttttccgatcctattaaacaaaagtttcccaacgacgcgaatgcagagagcgccagtaacaagttgcaggaattgcagccagacgttccgccatcctctggtcgatcttaa

SEQ ID NO: 26 - protein, 414 aa, synthetic construct
  source 1..414: note = CPB positioning fusion functional protein RCPB-PPKEX2
ASGHSYTKYNKWETIEAWIQQVATDNPDLVTQSVIGTTFEGRNMYVLKIGKTRPNKPAIFIDCGFHAREWISPAFCQWFVREAVRTYNQEIHMKQLLDELDFYVLPVVNIDGYVYTWTKDRMWRKTRSTMAGSSCLGVRPNRNFNAGWCEVGASRSPCSETYCGPAPESEKETKALADFIRNNLSTIKAYLTIHSYSQMMLYPYSYDYKLPENYEELNALVKGAAKELATLHGTKYTYGPGATTIYPAAGGSDDWSYDQGIKYSFTFELRDTGFFGFLLPESQIRQTCEETMLAVKYIANYVREHLYGGSGSGSGGSYLAFLLGLGFLICIIFLFTNRNKLERRQRRNRRDEYEFDLIPADDDFDTEEDQEANSQFTLDSDAELMFEDTSQREASPHEYQDSLGSNEHPKRAAL

SEQ ID NO: 27 - DNA, 1245 bp, synthetic construct
  source 1..1245: mol_type = other DNA; note = DNA sequence encoding RCPB-PPKEX2
gcaagcggtcactcgtacacaaagtataacaaatgggaaactatcgaggcctggattcaacaagtagccacggataaccctgatttagtcacgcaatcggtcatagggacaaccttcgagggcagaaacatgtacgtattaaagataggaaagactcgtcccaataaacctgctatttttatcgactgtggcttccacgctagagaatggattagccctgccttctgccaatggttcgtgagggaagcagtacggacgtacaaccaggaaattcatatgaagcaactgctcgacgaattagatttctatgttttaccggtagttaacatcgatggctacgtttacacatggacaaaagaccgtatgtggcggaagactagatcgacgatggcaggctcatcctgtctgggtgtgcgtccgaataggaacttcaatgcgggttggtgtgaagtgggggcgtcccgctctccctgttcagagacatactgcggacctgccccagaatccgaaaaagagacgaaagctcttgctgattttattaggaacaacctaagtaccattaaagcatacttaaccatccatagttacagccagatgatgctgtatccctattcctacgactataagctaccggagaactatgaagaactcaatgctttagttaaaggagcggccaaggagttggcgacattgcatggaacgaagtacacttatggtccaggggccactaccatctatccggcagctggtggatcagacgactggagttatgaccaaggtataaagtactctttcacctttgaattacgtgatactggtttttttggctttctgcttccagagtcacagatccgccagacttgcgaggaaaccatgcttgcggtgaagtatatagctaattacgtccgtgaacatctatacggcggatccgggtcggggagtggtgggagttatctagcatttttgctagggctcggcttcctgatctgcataatattcttgtttaccaaccgcaataaattggaacgaaggcagcgacgaaatcggcgagacgaatatgagtttgacctcattccggcggatgatgattttgatacggaggaggaccaggaggccaatagccaattcacattggactctgacgcggaacttatgttcgaagatacgtcacagagagaggcctcgccccacgagtatcaagattctctgggatctaatgaacacccaaaacgggctgcactttaa

SEQ ID NO: 28 - protein, 453 aa, synthetic construct
  source 1..453: note = CPB positioning fusion functional protein RCPB-SCKEX2
ASGHSYTKYNKWETIEAWIQQVATDNPDLVTQSVIGTTFEGRNMYVLKIGKTRPNKPAIFIDCGFHAREWISPAFCQWFVREAVRTYNQEIHMKQLLDELDFYVLPVVNIDGYVYTWTKDRMWRKTRSTMAGSSCLGVRPNRNFNAGWCEVGASRSPCSETYCGPAPESEKETKALADFIRNNLSTIKAYLTIHSYSQMMLYPYSYDYKLPENYEELNALVKGAAKELATLHGTKYTYGPGATTIYPAAGGSDDWSYDQGIKYSFTFELRDTGFFGFLLPESQIRQTCEETMLAVKYIANYVREHLYGGSGSGSGGSYFLTIFLIGATFLVLYFMFFMKSRRRIRRSRAETYEFDIIDTDSEYDSTLDNGTSGITEPEEVEDFDFDLSDEDHLASLSSSENGDAEHTIDSVLTNENPFSDPIKQKFPNDANAESASNKLQELQPDVPPSSGRS

SEQ ID NO: 29 - DNA, 1362 bp, synthetic construct
  source 1..1362: mol_type = other DNA; note = DNA sequence encoding RCPB-SCKEX2
gcaagcggtcactcgtacacaaagtataacaaatgggaaactatcgaggcctggattcaacaagtagccacggataaccctgatttagtcacgcaatcggtcatagggacaaccttcgagggcagaaacatgtacgtattaaagataggaaagactcgtcccaataaacctgctatttttatcgactgtggcttccacgctagagaatggattagccctgccttctgccaatggttcgtgagggaagcagtacggacgtacaaccaggaaattcatatgaagcaactgctcgacgaattagatttctatgttttaccggtagttaacatcgatggctacgtttacacatggacaaaagaccgtatgtggcggaagactagatcgacgatggcaggctcatcctgtctgggtgtgcgtccgaataggaacttcaatgcgggttggtgtgaagtgggggcgtcccgctctccctgttcagagacatactgcggacctgccccagaatccgaaaaagagacgaaagctcttgctgattttattaggaacaacctaagtaccattaaagcatacttaaccatccatagttacagccagatgatgctgtatccctattcctacgactataagctaccggagaactatgaagaactcaatgctttagttaaaggagcggccaaggagttggcgacattgcatggaacgaagtacacttatggtccaggggccactaccatctatccggcagctggtggatcagacgactggagttatgaccaaggtataaagtactctttcacctttgaattacgtgatactggtttttttggctttctgcttccagagtcacagatccgccagacttgcgaggaaaccatgcttgcggtgaagtatatagctaattacgtccgtgaacatctatacggcggatccgggtcggggagtggtgggagttatttcctcacaatattcttaataggcgcaacgtttttagtgctgtattttatgtttttcatgaaatcaaggcggagaatccggcgttcacgcgcggagacctacgagttcgacatcatagatactgactcggaatacgattcaaccctggataacgggacctcgggtattactgaacccgaggaggtagaggatttcgatttcgacctctctgacgaagatcatctagccagtctatcgtccagtgaaaatggagatgctgaacacacaatcgacagcgtccttacgaatgagaacccgttttccgatcctattaaacaaaagtttcccaacgacgcgaatgcagagagcgccagtaacaagttgcaggaattgcagccagacgttccgccatcctctggtcgatcttaa

SEQ ID NO: 30 - protein, 522 aa, synthetic construct
  source 1..522: note = Repeat tandem sequence 3A5D29N-9
EAGKSGDRGESGPAGPAGAPGPAGSRGAPGPQGPRGDKGETGERGAAGIKGHRGLEKREAGKSGDRGESGPAGPAGAPGPAGSRGAPGPQGPRGDKGETGERGAAGIKGHRGLEKREAGKSGDRGESGPAGPAGAPGPAGSRGAPGPQGPRGDKGETGERGAAGIKGHRGLEKREAGKSGDRGESGPAGPAGAPGPAGSRGAPGPQGPRGDKGETGERGAAGIKGHRGLEKREAGKSGDRGESGPAGPAGAPGPAGSRGAPGPQGPRGDKGETGERGAAGIKGHRGLEKREAGKSGDRGESGPAGPAGAPGPAGSRGAPGPQGPRGDKGETGERGAAGIKGHRGLEKREAGKSGDRGESGPAGPAGAPGPAGSRGAPGPQGPRGDKGETGERGAAGIKGHRGLEKREAGKSGDRGESGPAGPAGAPGPAGSRGAPGPQGPRGDKGETGERGAAGIKGHRGLEKREAGKSGDRGESGPAGPAGAPGPAGSRGAPGPQGPRGDKGETGERGAAGIKGHRGLEKR

SEQ ID NO: 31 - protein, 58 aa, synthetic construct
  source 1..58: note = Small protein sequence produced by Kex2 cleavage of 3A5D29N-9
EAGKSGDRGESGPAGPAGAPGPAGSRGAPGPQGPRGDKGETGERGAAGIKGHRGLEKR

SEQ ID NO: 32 - protein, 54 aa, synthetic construct
  source 1..54: note = Recombinant small-molecule collagen 3A5D29N
GKSGDRGESGPAGPAGAPGPAGSRGAPGPQGPRGDKGETGERGAAGIKGHRGLE

SEQ ID NO: 33 - protein, 536 aa, synthetic construct
  source 1..536: note = Repeat tandem sequence 17S28-8
EAGVPGSVGPKGSSGSPGPQGPPGPVGLQGLRGEVGLPGVKGDKGPMGPPGPKGDQGEKGPRGLEKREAGVPGSVGPKGSSGSPGPQGPPGPVGLQGLRGEVGLPGVKGDKGPMGPPGPKGDQGEKGPRGLEKREAGVPGSVGPKGSSGSPGPQGPPGPVGLQGLRGEVGLPGVKGDKGPMGPPGPKGDQGEKGPRGLEKREAGVPGSVGPKGSSGSPGPQGPPGPVGLQGLRGEVGLPGVKGDKGPMGPPGPKGDQGEKGPRGLEKREAGVPGSVGPKGSSGSPGPQGPPGPVGLQGLRGEVGLPGVKGDKGPMGPPGPKGDQGEKGPRGLEKREAGVPGSVGPKGSSGSPGPQGPPGPVGLQGLRGEVGLPGVKGDKGPMGPPGPKGDQGEKGPRGLEKREAGVPGSVGPKGSSGSPGPQGPPGPVGLQGLRGEVGLPGVKGDKGPMGPPGPKGDQGEKGPRGLEKREAGVPGSVGPKGSSGSPGPQGPPGPVGLQGLRGEVGLPGVKGDKGPMGPPGPKGDQGEKGPRGLEKR

SEQ ID NO: 34 - protein, 67 aa, synthetic construct
  source 1..67: note = Small protein sequence produced by Kex2 cleavage of 17S28-8
EAGVPGSVGPKGSSGSPGPQGPPGPVGLQGLRGEVGLPGVKGDKGPMGPPGPKGDQGEKGPRGLEKR

SEQ ID NO: 35 - protein, 63 aa, synthetic construct
  source 1..63: note = Recombinant small-molecule collagen 17S28
GVPGSVGPKGSSGSPGPQGPPGPVGLQGLRGEVGLPGVKGDKGPMGPPGPKGDQGEKGPRGLE

SEQ ID NO: 36 - protein, 540 aa, synthetic construct
  source 1..540: note = Repeat tandem sequence 17S1N6-6
EAGPPGSGEKGERGAAGEPGPHGPPGVPGSVGPKGSSGSPGPQGPPGPVGLQGLRGEVGLPGVKGDKGPMGPPGPKGDQGEKGPRGLEKREAGPPGSGEKGERGAAGEPGPHGPPGVPGSVGPKGSSGSPGPQGPPGPVGLQGLRGEVGLPGVKGDKGPMGPPGPKGDQGEKGPRGLEKREAGPPGSGEKGERGAAGEPGPHGPPGVPGSVGPKGSSGSPGPQGPPGPVGLQGLRGEVGLPGVKGDKGPMGPPGPKGDQGEKGPRGLEKREAGPPGSGEKGERGAAGEPGPHGPPGVPGSVGPKGSSGSPGPQGPPGPVGLQGLRGEVGLPGVKGDKGPMGPPGPKGDQGEKGPRGLEKREAGPPGSGEKGERGAAGEPGPHGPPGVPGSVGPKGSSGSPGPQGPPGPVGLQGLRGEVGLPGVKGDKGPMGPPGPKGDQGEKGPRGLEKREAGPPGSGEKGERGAAGEPGPHGPPGVPGSVGPKGSSGSPGPQGPPGPVGLQGLRGEVGLPGVKGDKGPMGPPGPKGDQGEKGPRGLEKR

SEQ ID NO: 37 - protein, 90 aa, synthetic construct
  source 1..90: note = Small protein sequence produced by Kex2 cleavage of 17S1N6-6
EAGPPGSGEKGERGAAGEPGPHGPPGVPGSVGPKGSSGSPGPQGPPGPVGLQGLRGEVGLPGVKGDKGPMGPPGPKGDQGEKGPRGLEKR

SEQ ID NO: 38 - protein, 86 aa, synthetic construct
  source 1..86: note = Recombinant small-molecule collagen 17S1N6
GPPGSGEKGERGAAGEPGPHGPPGVPGSVGPKGSSGSPGPQGPPGPVGLQGLRGEVGLPGVKGDKGPMGPPGPKGDQGEKGPRGLE

SEQ ID NO: 39 - protein, 528 aa, synthetic construct
  source 1..528: note = Repeat tandem sequence 17S1N7-7
EAGPPGSGEKGERGAAGEPGPHGPPGVPGSVGPKGSSGSPGPQGPPGPVGLQGLRGEVGLPGVKGDKGPMGPPGPKGDQGEKGPRGKREAGPPGSGEKGERGAAGEPGPHGPPGVPGSVGPKGSSGSPGPQGPPGPVGLQGLRGEVGLPGVKGDKGPMGPPGPKGDQGEKGPRGKREAGPPGSGEKGERGAAGEPGPHGPPGVPGSVGPKGSSGSPGPQGPPGPVGLQGLRGEVGLPGVKGDKGPMGPPGPKGDQGEKGPRGKREAGPPGSGEKGERGAAGEPGPHGPPGVPGSVGPKGSSGSPGPQGPPGPVGLQGLRGEVGLPGVKGDKGPMGPPGPKGDQGEKGPRGKREAGPPGSGEKGERGAAGEPGPHGPPGVPGSVGPKGSSGSPGPQGPPGPVGLQGLRGEVGLPGVKGDKGPMGPPGPKGDQGEKGPRGKREAGPPGSGEKGERGAAGEPGPHGPPGVPGSVGPKGSSGSPGPQGPPGPVGLQGLRGEVGLPGVKGDKGPMGPPGPKGDQGEKGPRGKR

SEQ ID NO: 40 - protein, 88 aa, synthetic construct
  source 1..88: note = Small protein sequence produced by Kex2 cleavage of 17S1N7-7
EAGPPGSGEKGERGAAGEPGPHGPPGVPGSVGPKGSSGSPGPQGPPGPVGLQGLRGEVGLPGVKGDKGPMGPPGPKGDQGEKGPRGKR

SEQ ID NO: 41 - protein, 84 aa, synthetic construct
  source 1..84: note = Recombinant small-molecule collagen 17S1N7
GPPGSGEKGERGAAGEPGPHGPPGVPGSVGPKGSSGSPGPQGPPGPVGLQGLRGEVGLPGVKGDKGPMGPPGPKGDQGEKGPRG

SEQ ID NO: 42 - protein, 595 aa, synthetic construct
  source 1..595: note = Repeat tandem sequence 17S1NK-7
EAGPPGSGEKGERGAAGEPGPHGPPGVPGSVGPKGSSGSPGPQGPPGPVGLQGLRGEVGLPGVKGDKGPMGPPGPKGDQGEKGKREAGPPGSGEKGERGAAGEPGPHGPPGVPGSVGPKGSSGSPGPQGPPGPVGLQGLRGEVGLPGVKGDKGPMGPPGPKGDQGEKGKREAGPPGSGEKGERGAAGEPGPHGPPGVPGSVGPKGSSGSPGPQGPPGPVGLQGLRGEVGLPGVKGDKGPMGPPGPKGDQGEKGKREAGPPGSGEKGERGAAGEPGPHGPPGVPGSVGPKGSSGSPGPQGPPGPVGLQGLRGEVGLPGVKGDKGPMGPPGPKGDQGEKGKREAGPPGSGEKGERGAAGEPGPHGPPGVPGSVGPKGSSGSPGPQGPPGPVGLQGLRGEVGLPGVKGDKGPMGPPGPKGDQGEKGKREAGPPGSGEKGERGAAGEPGPHGPPGVPGSVGPKGSSGSPGPQGPPGPVGLQGLRGEVGLPGVKGDKGPMGPPGPKGDQGEKGKREAGPPGSGEKGERGAAGEPGPHGPPGVPGSVGPKGSSGSPGPQGPPGPVGLQGLRGEVGLPGVKGDKGPMGPPGPKGDQGEKGKR

SEQ ID NO: 43 - protein, 85 aa, synthetic construct
  source 1..85: note = Small protein sequence produced by Kex2 cleavage of 17S1NK-7
EAGPPGSGEKGERGAAGEPGPHGPPGVPGSVGPKGSSGSPGPQGPPGPVGLQGLRGEVGLPGVKGDKGPMGPPGPKGDQGEKGKR

SEQ ID NO: 44 - protein, 84 aa, synthetic construct; identical to SEQ ID NO: 41
  source 1..84: note = Recombinant small-molecule collagen 17S1NK

SEQ ID NO: 45 - protein, 510 aa, synthetic construct
  source 1..510: note = Repeat tandem sequence 3A5D15D-5
DGNPGSDGLPGRDGSPGGKGDRGENGSPGAPGAPGHPGPPGPVGPAGKSGDRGESGPAGPAGAPGPAGSRGAPGPQGPRGDKGETGERGAAGIKGHRGLEKRDGNPGSDGLPGRDGSPGGKGDRGENGSPGAPGAPGHPGPPGPVGPAGKSGDRGESGPAGPAGAPGPAGSRGAPGPQGPRGDKGETGERGAAGIKGHRGLEKRDGNPGSDGLPGRDGSPGGKGDRGENGSPGAPGAPGHPGPPGPVGPAGKSGDRGESGPAGPAGAPGPAGSRGAPGPQGPRGDKGETGERGAAGIKGHRGLEKRDGNPGSDGLPGRDGSPGGKGDRGENGSPGAPGAPGHPGPPGPVGPAGKSGDRGESGPAGPAGAPGPAGSRGAPGPQGPRGDKGETGERGAAGIKGHRGLEKRDGNPGSDGLPGRDGSPGGKGDRGENGSPGAPGAPGHPGPPGPVGPAGKSGDRGESGPAGPAGAPGPAGSRGAPGPQGPRGDKGETGERGAAGIKGHRGLEKR

SEQ ID NO: 46 - protein, 102 aa, synthetic construct
  source 1..102: note = Small protein sequence produced by Kex2 cleavage of 3A5D15D-5
DGNPGSDGLPGRDGSPGGKGDRGENGSPGAPGAPGHPGPPGPVGPAGKSGDRGESGPAGPAGAPGPAGSRGAPGPQGPRGDKGETGERGAAGIKGHRGLEKR

SEQ ID NO: 47 - protein, 100 aa, synthetic construct
  source 1..100: note = Recombinant small-molecule collagen 3A5D15D
DGNPGSDGLPGRDGSPGGKGDRGENGSPGAPGAPGHPGPPGPVGPAGKSGDRGESGPAGPAGAPGPAGSRGAPGPQGPRGDKGETGERGAAGIKGHRGLE

SEQ ID NO: 48 - protein, 520 aa, synthetic construct
  source 1..520: note = Repeat tandem sequence 3A5D15E-5
EADGNPGSDGLPGRDGSPGGKGDRGENGSPGAPGAPGHPGPPGPVGPAGKSGDRGESGPAGPAGAPGPAGSRGAPGPQGPRGDKGETGERGAAGIKGHRGLEKREADGNPGSDGLPGRDGSPGGKGDRGENGSPGAPGAPGHPGPPGPVGPAGKSGDRGESGPAGPAGAPGPAGSRGAPGPQGPRGDKGETGERGAAGIKGHRGLEKREADGNPGSDGLPGRDGSPGGKGDRGENGSPGAPGAPGHPGPPGPVGPAGKSGDRGESGPAGPAGAPGPAGSRGAPGPQGPRGDKGETGERGAAGIKGHRGLEKREADGNPGSDGLPGRDGSPGGKGDRGENGSPGAPGAPGHPGPPGPVGPAGKSGDRGESGPAGPAGAPGPAGSRGAPGPQGPRGDKGETGERGAAGIKGHRGLEKREADGNPGSDGLPGRDGSPGGKGDRGENGSPGAPGAPGHPGPPGPVGPAGKSGDRGESGPAGPAGAPGPAGSRGAPGPQGPRGDKGETGERGAAGIKGHRGLEKR

SEQ ID NO: 49 - protein, 104 aa, synthetic construct
  source 1..104: note = Small protein sequence produced by Kex2 cleavage of 3A5D15E-5
EADGNPGSDGLPGRDGSPGGKGDRGENGSPGAPGAPGHPGPPGPVGPAGKSGDRGESGPAGPAGAPGPAGSRGAPGPQGPRGDKGETGERGAAGIKGHRGLEKR

SEQ ID NO: 50 - protein, 100 aa, synthetic construct; identical to SEQ ID NO: 47
  source 1..100: note = Recombinant small-molecule collagen 3A5D15E

SEQ ID NO: 51 - protein, 570 aa, synthetic construct
  source 1..570: note = Repeat tandem sequence 3A5D15R-6
DGNPGSDGLPGRDGSPGGKGDRGENGSPGAPGAPGHPGPPGPVGPAGKSGDRGESGPAGPAGAPGPAGSRGAPGPQGPRGDKGETGERGAAGIKRDGNPGSDGLPGRDGSPGGKGDRGENGSPGAPGAPGHPGPPGPVGPAGKSGDRGESGPAGPAGAPGPAGSRGAPGPQGPRGDKGETGERGAAGIKRDGNPGSDGLPGRDGSPGGKGDRGENGSPGAPGAPGHPGPPGPVGPAGKSGDRGESGPAGPAGAPGPAGSRGAPGPQGPRGDKGETGERGAAGIKRDGNPGSDGLPGRDGSPGGKGDRGENGSPGAPGAPGHPGPPGPVGPAGKSGDRGESGPAGPAGAPGPAGSRGAPGPQGPRGDKGETGERGAAGIKRDGNPGSDGLPGRDGSPGGKGDRGENGSPGAPGAPGHPGPPGPVGPAGKSGDRGESGPAGPAGAPGPAGSRGAPGPQGPRGDKGETGERGAAGIKRDGNPGSDGLPGRDGSPGGKGDRGENGSPGAPGAPGHPGPPGPVGPAGKSGDRGESGPAGPAGAPGPAGSRGAPGPQGPRGDKGETGERGAAGIKR

SEQ ID NO: 52 - protein, 95 aa, synthetic construct
  source 1..95: note = Small protein sequence produced by Kex2 cleavage of 3A5D15R-6
DGNPGSDGLPGRDGSPGGKGDRGENGSPGAPGAPGHPGPPGPVGPAGKSGDRGESGPAGPAGAPGPAGSRGAPGPQGPRGDKGETGERGAAGIKR

SEQ ID NO: 53 - protein, 93 aa, synthetic construct
  source 1..93: note = Recombinant small-molecule collagen 3A5D15R
DGNPGSDGLPGRDGSPGGKGDRGENGSPGAPGAPGHPGPPGPVGPAGKSGDRGESGPAGPAGAPGPAGSRGAPGPQGPRGDKGETGERGAAGI

SEQ ID NO: 54 - protein, 582 aa, synthetic construct
  source 1..582: note = Repeat tandem sequence 3A5D15KR-6
DGNPGSDGLPGRDGSPGGKGDRGENGSPGAPGAPGHPGPPGPVGPAGKSGDRGESGPAGPAGAPGPAGSRGAPGPQGPRGDKGETGERGAAGIKGKRDGNPGSDGLPGRDGSPGGKGDRGENGSPGAPGAPGHPGPPGPVGPAGKSGDRGESGPAGPAGAPGPAGSRGAPGPQGPRGDKGETGERGAAGIKGKRDGNPGSDGLPGRDGSPGGKGDRGENGSPGAPGAPGHPGPPGPVGPAGKSGDRGESGPAGPAGAPGPAGSRGAPGPQGPRGDKGETGERGAAGIKGKRDGNPGSDGLPGRDGSPGGKGDRGENGSPGAPGAPGHPGPPGPVGPAGKSGDRGESGPAGPAGAPGPAGSRGAPGPQGPRGDKGETGERGAAGIKGKRDGNPGSDGLPGRDGSPGGKGDRGENGSPGAPGAPGHPGPPGPVGPAGKSGDRGESGPAGPAGAPGPAGSRGAPGPQGPRGDKGETGERGAAGIKGKRDGNPGSDGLPGRDGSPGGKGDRGENGSPGAPGAPGHPGPPGPVGPAGKSGDRGESGPAGPAGAPGPAGSRGAPGPQGPRGDKGETGERGAAGIKGKR

SEQ ID NO: 55 - protein, 97 aa, synthetic construct
  source 1..97: note = Small protein sequence produced by Kex2 cleavage of 3A5D15KR-6
DGNPGSDGLPGRDGSPGGKGDRGENGSPGAPGAPGHPGPPGPVGPAGKSGDRGESGPAGPAGAPGPAGSRGAPGPQGPRGDKGETGERGAAGIKGKR

SEQ ID NO: 56 - protein, 95 aa, synthetic construct
  source 1..95: note = Recombinant small-molecule collagen 3A5D15KR
DGNPGSDGLPGRDGSPGGKGDRGENGSPGAPGAPGHPGPPGPVGPAGKSGDRGESGPAGPAGAPGPAGSRGAPGPQGPRGDKGETGERGAAGIKG

SEQ ID NO: 57 - protein, 576 aa, synthetic construct
  source 1..576: note = Repeat tandem sequence 3A5D15EKR-6
DGNPGSDGLPGRDGSPGGKGDRGENGSPGAPGAPGHPGPPGPVGPAGKSGDRGESGPAGPAGAPGPAGSRGAPGPQGPRGDKGETGERGAAGIEKRDGNPGSDGLPGRDGSPGGKGDRGENGSPGAPGAPGHPGPPGPVGPAGKSGDRGESGPAGPAGAPGPAGSRGAPGPQGPRGDKGETGERGAAGIEKRDGNPGSDGLPGRDGSPGGKGDRGENGSPGAPGAPGHPGPPGPVGPAGKSGDRGESGPAGPAGAPGPAGSRGAPGPQGPRGDKGETGERGAAGIEKRDGNPGSDGLPGRDGSPGGKGDRGENGSPGAPGAPGHPGPPGPVGPAGKSGDRGESGPAGPAGAPGPAGSRGAPGPQGPRGDKGETGERGAAGIEKRDGNPGSDGLPGRDGSPGGKGDRGENGSPGAPGAPGHPGPPGPVGPAGKSGDRGESGPAGPAGAPGPAGSRGAPGPQGPRGDKGETGERGAAGIEKRDGNPGSDGLPGRDGSPGGKGDRGENGSPGAPGAPGHPGPPGPVGPAGKSGDRGESGPAGPAGAPGPAGSRGAPGPQGPRGDKGETGERGAAGIEKR

SEQ ID NO: 58 - protein, 96 aa, synthetic construct
  source 1..96: note = Small protein sequence produced by Kex2 cleavage of 3A5D15EKR-6
DGNPGSDGLPGRDGSPGGKGDRGENGSPGAPGAPGHPGPPGPVGPAGKSGDRGESGPAGPAGAPGPAGSRGAPGPQGPRGDKGETGERGAAGIEKR

SEQ ID NO: 59 - protein, 94 aa, synthetic construct
  source 1..94: note = Recombinant small-molecule collagen 3A5D15EKR
DGNPGSDGLPGRDGSPGGKGDRGENGSPGAPGAPGHPGPPGPVGPAGKSGDRGESGPAGPAGAPGPAGSRGAPGPQGPRGDKGETGERGAAGIE

SEQ ID NO: 60 - protein, 576 aa, synthetic construct
  source 1..576: note = Repeat tandem sequence 3A5D15G-6
DGNPGSDGLPGRDGSPGGKGDRGENGSPGAPGAPGHPGPPGPVGPAGKSGDRGESGPAGPAGAPGPAGSRGAPGPQGPRGDKGETGERGAAGIGKRDGNPGSDGLPGRDGSPGGKGDRGENGSPGAPGAPGHPGPPGPVGPAGKSGDRGESGPAGPAGAPGPAGSRGAPGPQGPRGDKGETGERGAAGIGKRDGNPGSDGLPGRDGSPGGKGDRGENGSPGAPGAPGHPGPPGPVGPAGKSGDRGESGPAGPAGAPGPAGSRGAPGPQGPRGDKGETGERGAAGIGKRDGNPGSDGLPGRDGSPGGKGDRGENGSPGAPGAPGHPGPPGPVGPAGKSGDRGESGPAGPAGAPGPAGSRGAPGPQGPRGDKGETGERGAAGIGKRDGNPGSDGLPGRDGSPGGKGDRGENGSPGAPGAPGHPGPPGPVGPAGKSGDRGESGPAGPAGAPGPAGSRGAPGPQGPRGDKGETGERGAAGIGKRDGNPGSDGLPGRDGSPGGKGDRGENGSPGAPGAPGHPGPPGPVGPAGKSGDRGESGPAGPAGAPGPAGSRGAPGPQGPRGDKGETGERGAAGIGKR

SEQ ID NO: 61 - protein, 96 aa, synthetic construct
  source 1..96: note = Small protein sequence produced by Kex2 cleavage of 3A5D15G-6
DGNPGSDGLPGRDGSPGGKGDRGENGSPGAPGAPGHPGPPGPVGPAGKSGDRGESGPAGPAGAPGPAGSRGAPGPQGPRGDKGETGERGAAGIGKR

SEQ ID NO: 62 - protein, 94 aa, synthetic construct
  source 1..94: note = Recombinant small-molecule collagen 3A5D15G
DGNPGSDGLPGRDGSPGGKGDRGENGSPGAPGAPGHPGPPGPVGPAGKSGDRGESGPAGPAGAPGPAGSRGAPGPQGPRGDKGETGERGAAGIG

SEQ ID NO: 63 - protein, 96 aa, synthetic construct
  source 1..96: note = Recombinant small-molecule collagen
GPPGPAGNTGAPGSPGVSGPKGDAGQPGEKGSPGAQGPQGVKGESGKPGANGLSGENGSPGAPGAPGHPGPPGPVGPAGKSGAPGPQGPRGDKGET

SEQ ID NO: 64 - protein, 500 aa, synthetic construct
  source 1..500: note = Repeat tandem sequence 3A5D16M-6
EAGPPGPAGNTGAPGSPGVSGPKGDAGQPGEKGSPGAQGPQGVKGESGKPGANGLSGENGSPGAPGAPGHPGPPGPVGPAGKSGAPGPQGPRGDKGLEKREAGPPGPAGNTGAPGSPGVSGPKGDAGQPGEKGSPGAQGPQGVKGESGKPGANGLSGENGSPGAPGAPGHPGPPGPVGPAGKSGAPGPQGPRGDKGLEKREAGPPGPAGNTGAPGSPGVSGPKGDAGQPGEKGSPGAQGPQGVKGESGKPGANGLSGENGSPGAPGAPGHPGPPGPVGPAGKSGAPGPQGPRGDKGLEKREAGPPGPAGNTGAPGSPGVSGPKGDAGQPGEKGSPGAQGPQGVKGESGKPGANGLSGENGSPGAPGAPGHPGPPGPVGPAGKSGAPGPQGPRGDKGLEKREAGPPGPAGNTGAPGSPGVSGPKGDAGQPGEKGSPGAQGPQGVKGESGKPGANGLSGENGSPGAPGAPGHPGPPGPVGPAGKSGAPGPQGPRGDKGLEKR

SEQ ID NO: 65 - protein, 100 aa, synthetic construct
  source 1..100: note = Small protein sequence produced by Kex2 cleavage of 3A5D16M-6
EAGPPGPAGNTGAPGSPGVSGPKGDAGQPGEKGSPGAQGPQGVKGESGKPGANGLSGENGSPGAPGAPGHPGPPGPVGPAGKSGAPGPQGPRGDKGLEKR

SEQ ID NO: 66 - protein, 96 aa, synthetic construct
  source 1..96: note = Recombinant small-molecule collagen 3A5D16M
GPPGPAGNTGAPGSPGVSGPKGDAGQPGEKGSPGAQGPQGVKGESGKPGANGLSGENGSPGAPGAPGHPGPPGPVGPAGKSGAPGPQGPRGDKGLE

SEQ ID NO: 67 - protein, 39 aa, synthetic construct
  source 1..39: note = Recombinant small-molecule collagen
GSPGAPGAPGHPGPPGPVGPAGKSGAPGPQGPRGDKGET

SEQ ID NO: 68 - protein, 516 aa, synthetic construct
  source 1..516: note = Repeat tandem sequence 3A5D15M-12
EAGSPGAPGAPGHPGPPGPVGPAGKSGAPGPQGPRGDKGLEKREAGSPGAPGAPGHPGPPGPVGPAGKSGAPGPQGPRGDKGLEKREAGSPGAPGAPGHPGPPGPVGPAGKSGAPGPQGPRGDKGLEKREAGSPGAPGAPGHPGPPGPVGPAGKSGAPGPQGPRGDKGLEKREAGSPGAPGAPGHPGPPGPVGPAGKSGAPGPQGPRGDKGLEKREAGSPGAPGAPGHPGPPGPVGPAGKSGAPGPQGPRGDKGLEKREAGSPGAPGAPGHPGPPGPVGPAGKSGAPGPQGPRGDKGLEKREAGSPGAPGAPGHPGPPGPVGPAGKSGAPGPQGPRGDKGLEKREAGSPGAPGAPGHPGPPGPVGPAGKSGAPGPQGPRGDKGLEKREAGSPGAPGAPGHPGPPGPVGPAGKSGAPGPQGPRGDKGLEKREAGSPGAPGAPGHPGPPGPVGPAGKSGAPGPQGPRGDKGLEKREAGSPGAPGAPGHPGPPGPVGPAGKSGAPGPQGPRGDKGLEKR

SEQ ID NO: 69 - protein, 43 aa, synthetic construct
  source 1..43: note = Small protein sequence produced by Kex2 cleavage of 3A5D15M-12
EAGSPGAPGAPGHPGPPGPVGPAGKSGAPGPQGPRGDKGLEKR

SEQ ID NO: 70 - protein, 39 aa, synthetic construct
  source 1..39: note = Recombinant small-molecule collagen 3A5D15M
GSPGAPGAPGHPGPPGPVGPAGKSGAPGPQGPRGDKGLE

SEQ ID NO: 71 - DNA, 1569 bp, synthetic construct
  source 1..1569: mol_type = other DNA; note = DNA sequence encoding 3A5D29N-9
gaagctggaaagtccggcgaccggggagagtcagggcctgcagggcctgctggtgccccaggaccggccggcagtagaggtgctcctggtcctcaaggaccacggggcgacaaaggtgaaacaggtgaacgaggtgcggcaggtataaaagggcacagagggctagaaaagcgggaagcaggaaaaagtggcgatcgcggggaatcaggtcccgcggggccggcgggtgcgcccggaccggcggggtccagaggtgcccctggaccgcagggacctcggggtgacaaaggtgaaactggggaaaggggggctgcgggcataaagggacaccgcggactcgagaagagagaggcaggtaaaagtggggatagaggcgaatctggtccggcaggaccagcgggcgcccccggtcctgctggatcacgaggtgccccgggtccgcaaggtcctaggggtgacaaaggcgagacgggcgaacgaggggcagcaggaattaaaggccaccgagggctggagaagcgggaagcaggtaaatcaggagataggggggaaagcggaccggccggacccgctggtgcgccgggacctgctggatcgagaggtgcaccgggtccccaagggcctcgtggagataaaggggagaccggggagcgcggggctgcagggattaagggacaccgcggcttggagaagcgagaggctggtaaaagcggcgaccgcggcgaatcgggtccggcgggtcccgcgggcgcacctgggcctgctgggtctaggggagcgccagggcctcaaggtcctcgcggtgacaagggagaaacaggcgagcgtggggcagcgggcattaaaggtcatcgtgggttagaaaagcgtgaggctggcaaatctggcgatcgcggggagagcggtccagcaggtccggctggtgctccaggtccagctggtagccgtggcgccccaggtcctcaaggtcctcgtggcgacaaaggggagaccggcgagcgtggagcggcaggcatcaaaggtcatcgtggacttgaaaagagggaggcgggaaagtcgggcgatcggggtgaatccggcccagcgggtcctgctggagccccaggccccgctggatcgcggggcgcacctggcccccaaggaccgcgtggggataaaggggagactggcgagagaggcgccgccggaatcaaaggtcaccggggattagaaaagagggaggcagggaagtcgggtgatcgaggcgaatcaggtcctgctggacccgctggcgcgccgggtcctgctggtagcagaggagcccctgggcctcaaggcccgaggggtgataagggtgaaaccggagaacgaggcgccgctggtataaagggacatcgtggactcgagaagcgagaagcggggaaaagtggggacagaggagagtctggtcctgccggacccgccggtgctcctggtccagcaggctcccgcggcgcgcctggtccgcaaggtcctaggggagacaaaggagaaacgggcgagcgaggcgccgccgggatcaaggggcatcgggggttggagaagaggtaa

SEQ ID NO: 72 - DNA, 1611 bp, synthetic construct
  source 1..1611: mol_type = other DNA; note = DNA sequence encoding 17S28-8
gaggccggtgtacccggaagcgtggggccgaagggcagctcgggttcaccaggcccacaggggccaccaggcccggtaggcctacaaggtttgcgcggtgaggtggggttacccggagtaaaaggtgataaggggcctatggggcctcccggtcctaaaggcgaccagggtgaaaagggtccgcggggactggagaaaagagaagcgggtgttccagggtcggttggtcctaagggaagttcgggttctccggggccgcaaggtcctccaggtcccgtcggtttacagggcctacgtggagaagtcggactccccggagttaagggcgataagggacccatgggtcctcctggtcccaaaggtgaccaaggcgagaaaggcccaaggggactcgagaagcgggaagcgggagtccctggctccgttggccctaagggaagttccggaagtccgggaccgcaaggtcctcctggccctgtcggcctccaaggtttgaggggagaggttggactccccggcgtcaagggcgacaaaggccctatggggccacctgggcctaagggcgaccaaggcgagaaaggccctcgcgggcttgagaagcgtgaagctggagtgcctgggtcagtaggcccaaaaggatcgtccggatcaccgggacctcaggggccaccgggtcctgtaggtctacagggcctcaggggcgaggtaggtttacctggagtcaagggagataagggacctatggggccgccaggtccgaaaggcgatcaaggggaaaaagggcctcgtggactagaaaaacgtgaggcaggcgtccctggatcggttggtcctaaaggttcttcaggtagtcccggtccccagggacctcccgggccggtagggctacagggcttacgaggggaggtgggcctcccaggggttaaaggggataaaggtcctatgggtcctccgggtccaaaaggtgatcagggtgagaagggtcctcgtgggctggaaaagagagaagcaggtgttccaggctctgttggaccgaaggggtcttctggaagccctggtcctcaaggtcctcctggtccggtcggacttcagggattgcgaggcgaggtaggtctgcccggggttaagggtgacaaagggccaatgggaccgccagggccgaaaggcgaccaaggtgaaaaaggccctcgaggtctggaaaaaagagaagctggagtaccagggagcgtcggccccaaaggaagttcggggtcccctggaccgcaagggccaccaggtcccgtagggttacaaggtctgcggggggaggttgggcttcccggagttaaaggtgataagggaccaatgggtcctcccggtccaaagggtgatcaaggagagaaaggaccgcgcgggctagaaaagagggaggccggtgtcccaggtagcgttggtcctaagggcagctcaggctccccaggaccccaagggccgccggggcctgtggggttgcaaggtttgcgaggagaagtgggccttcccggggtgaagggggacaagggacctatgggaccacccggtcccaaaggtgaccagggtgaaaagggtcctcgtggacttgaaaaaagataa

SEQ ID NO: 73 - DNA, 1623 bp, synthetic construct
  source 1..1623: mol_type = other DNA; note = DNA sequence encoding 17S1N6-6
gaagcgggacctcccggcagtggtgaaaagggcgaacgaggcgcagccggagagcctggacctcatgggcctccgggcgtcccgggaagtgttggtcctaaaggtagctccggatctccaggtccacagggaccacctggcccggtaggccttcaaggactgagaggtgaggtcggccttccaggcgtgaagggcgataaaggtcctatgggtccacctggacccaagggagatcagggggagaaagggccgaggggcttagaaaaacgcgaagcagggcctcctgggagcggagaaaagggcgagcgcggagccgcaggcgagccaggtcctcatggtcctccaggagtgcctgggtccgtcggcccaaaggggtcttctggttcgcctgggcctcaaggaccaccaggtcccgttggtttgcagggtctgcgtggagaagtgggccttccgggagttaagggcgacaagggtcctatggggcctccggggccgaagggcgatcagggcgaaaaaggcccccgcgggttagaaaaaagagaggcaggaccacccggctcaggtgagaagggtgaaagaggagccgctggggagccaggaccacacggcccccccggagtcccgggatctgttggacccaaaggttcttctgggagcccgggtccccagggaccgccaggcccagtaggtctacaaggactcagaggggaggtgggtctaccgggggtcaaaggagataagggtcctatgggtcctcccggtccaaaaggggaccaaggagagaagggacctcggggtttggaaaaacgggaagctggtcctcccggtagcggtgagaaaggcgagcgaggtgctgctggggaaccggggccacacggtcctcctggcgtgcccggctcggtcggacctaaaggttcttctggttctccgggtcctcaggggccgcctggtcctgtcgggcttcaaggtctccgcggtgaggttgggctccccggtgtcaagggagacaaagggccgatggggccgccaggtcccaagggagaccagggagaaaaaggtcctcgtgggttagaaaaacgggaggcgggaccgcctggttccggcgagaagggggaacgaggcgcggccggggaaccaggaccccatggaccgccaggtgttccggggtccgtaggtccgaaaggctcatcgggttcgcctggcccacaaggaccaccaggcccagtgggcctacaaggtctgaggggggaagttgggctccctggcgtaaagggagacaaagggccgatgggtcctcctggacccaaaggtgaccaaggagaaaaaggtccgaggggcttagagaaacgtgaagcaggtccgccaggttcaggtgagaagggggaacgtggagctgccggggagcctggcccgcacggccctcccggcgttcccggctcagttggaccaaagggatcgagtggaagtcctggtcctcaaggcccacctggtccagtaggtctacagggcttgaggggggaggtaggactgccgggcgtaaagggcgataagggtcccatgggtcctccagggcctaaaggtgatcagggggagaagggtccccgagggttggagaagcggtaa

SEQ ID NO: 74 - DNA, 1851 bp, synthetic construct
  source 1..1851: mol_type = other DNA; note = DNA sequence encoding 17S1N7-7
gaggcaggtcctccgggttctggtgagaagggcgaaaggggagctgcgggagaacctggcccacatggtcctcctggtgtacccgggtcggttggtcctaaagggtcttcaggctcccccggtccccagggaccaccgggtcctgttggtctccagggcctgcgaggggaggtgggacttccgggagtcaaaggagacaaaggtcctatgggtcctcctggtcctaaaggcgatcagggtgaaaagggaccgcgaggcaagagagaggctggtcctcccggaagcggtgagaagggtgagcgaggggctgctggagagccaggtccacacggacctcccggtgttcccggcagcgtaggcccaaaagggtcgtctgggtccccggggccacaaggtccccctggacccgtagggttgcaaggcctacggggagaagtaggattaccgggtgtgaagggcgacaaaggtcctatgggaccccccggtcccaagggtgatcagggtgagaagggtccgaggggtaaacgcgaagctggtccaccaggatctggcgaaaagggagaacgtggtgctgcgggagagcctgggccacacggtcccccgggagtacctgggagtgttgggccgaagggcagtagtggctcaccggggccgcaaggcccccccggaccggtaggactacaaggcttacggggggaggtaggtcttcctggggtgaagggggataaaggtcctatgggaccacccggcccaaaaggggaccagggagagaaagggccacgcggaaaaagggaggcaggcccaccggggtcgggtgaaaagggtgaacgcggagcggcgggggaaccggggcctcatgggccaccgggcgtgccaggttcggttggtcctaagggttcaagcggatctccaggcccgcagggacctcctggacccgttgggcttcagggactgcgtggcgaggtcggtctgcccggcgtcaagggagacaagggtcctatgggtcctccgggtccaaagggagatcagggtgagaagggacccagagggaaaagagaagctggccctccggggtccggggagaagggggaacgtggggcagccggtgagccgggacctcacggcccaccaggcgtgcctgggtccgttggcccaaaggggtcctcgggctcgccaggccctcagggaccaccgggtccagtcggattacaaggtttgcggggagaggttgggctccctggagttaaaggtgacaaaggccctatgggtcccccgggtcctaaaggcgaccaaggcgaaaaaggaccgagagggaaacgtgaagcaggtccacctgggtcaggtgagaaaggcgagcgcggggccgccggggaaccggggccacacggtcctcctggcgtccccggcagcgtcggcccgaaaggaagttctggaagtccgggaccacagggtccgcccggtcctgtagggctacaaggtttaagaggcgaagtgggactccctggcgtgaaaggtgacaaaggccccatgggaccaccaggtcctaaaggggatcagggagaaaaggggcctaggggtaaacgagaggcaggtccccccgggagcggagaaaagggtgagcgaggggccgccggtgaaccaggcccgcatggtccaccaggcgtccccggatcagtcggaccaaaaggcagttctggctcacctggaccgcaaggtccgcctggacctgtaggacttcaaggcctgcgtggtgaagttgggttgcctggggttaagggggataagggtcctatgggtccccctgggccaaaaggggatcaaggcgaaaagggtccccggggaaaaaggtaa

SEQ ID NO: 75 - DNA, 1788 bp, synthetic construct
  source 1..1788: mol_type = other DNA; note = DNA sequence encoding 17S1NK-7
gaagcaggtccgccagggagcggtgaaaaaggagaacgcggagcggcgggcgagccaggcccgcacgggccgcccggtgttcccggctctgttggaccgaaaggtagttctggttcacccggacctcaaggtcctcctgggcctgttggacttcaggggcttagaggtgaggtcggactccctggtgtgaaaggggataaagggcctatgggtcctcctgggccaaaaggggaccagggagagaaggggaagagggaggctggtcctccaggatcgggggaaaaaggagaacgtggagctgccggcgagccggggccacacggtccaccgggcgtccccgggtccgtgggacccaagggctcatcaggatcgccaggaccgcagggtcctccaggtcctgttgggttgcaggggttacgtggagaagtgggtctccccggtgttaaaggtgacaagggtcccatgggaccccccggtcctaaaggagaccaaggagagaaaggtaaacgagaggccgggccacctgggtccggcgagaagggcgaacgtggtgccgctggcgagcccgggcctcacggtccaccgggagtgcccgggtcagtaggcccgaaaggaagttccggaagtccaggtcctcaaggtcccccgggacctgtaggcctgcaagggttgcgtggtgaggtcggtctccctggggttaagggtgacaaaggtcctatgggtcctcccggacctaaaggggatcaaggggaaaaaggaaaacgagaggctggaccaccaggttctggcgaaaaaggtgagcgaggcgccgcgggcgaacccggcccgcatggccccccaggcgtaccaggctctgtgggtccgaagggctcgagcggttcacctggacctcaagggccacctggaccggttgggctacaaggcctacggggggaggtgggactaccgggcgtcaaaggtgacaaaggcccgatgggaccaccaggccctaagggagatcagggcgagaagggtaagagagaagcaggaccgccgggaagcggcgaaaaaggtgagcgcggagcagcaggggaacccgggccgcatggtccccctggcgtacctggtagcgttggtcctaaagggtcgtcgggttccccaggtcctcagggtccccctggtcctgtcggtctgcaagggttaaggggggaagtaggattaccgggcgtgaaaggagataaaggtcctatggggccacctggtcctaagggcgaccagggtgagaagggtaagcgcgaagctggcccgccgggtagtggtgagaaaggcgagcggggggcagcgggcgaaccaggtcctcatggtcctcctggtgtgccaggctccgtcggccctaagggatctagcggaagcccgggtccgcagggaccaccaggtcctgttggccttcaagggttgagaggtgaagtcggcttaccaggggtcaaaggtgataaaggcccgatgggtccacctgggcctaagggggatcagggggagaagggaaagcgggaagccggtccccccggaagtggagaaaagggggagaggggggctgcaggtgaacctgggcctcacggaccaccgggtgttccaggatcagttggacccaagggtagttcgggatctcctggccctcaaggcccccctggtcctgtaggacttcaagggctgcggggggaggtaggtctccctggtgtcaaaggagacaaaggaccgatgggtcctcctggtcctaagggagatcaaggagaaaaagggaagcgctaa

SEQ ID NO: 76 - DNA, 1533 bp, synthetic construct
  source 1..1533: mol_type = other DNA; note = DNA sequence encoding 3A5D15D-5
gatgggaacccggggtcggacggcctgccgggtcgcgacggctcaccaggtggcaaaggcgaccgtggtgagaatggatctccgggagcacccggtgcccctggacatcctggtccccccgggcctgtcggtcctgctggcaagtcgggtgatagaggagaatccgggcctgccggtcctgctggggcaccagggccagcaggaagccgtggggctcccggtcctcaaggtccccggggggacaagggtgagaccggagaacgcggagctgcgggaatcaaggggcatcgcggcttagagaaacgtgatggcaacccgggctctgacgggcttcccggtcgggacggcagccccggtgggaaaggtgatcgaggggaaaacggctcgcctggggctccaggtgcccccggccaccctggaccgccaggtcctgtcggccctgccggtaagagcggagatcgaggtgaatcaggacctgccggcccagccggtgctcctggtccagctggaagccgtggtgctcccggcccgcagggtcctcgtggcgataaaggcgagacgggtgaacggggcgcagccggaattaaaggacacagaggtcttgaaaagagggatggaaacccaggctcagatggtctaccaggcagggacgggtcacccggaggaaagggtgatcggggcgaaaacggctccccgggagcgccaggtgcccctgggcatcccgggccacccggaccggtgggtcccgcagggaaatcgggggataggggcgagtctggaccagcggggcctgcgggagcacctgggccagcaggtagtaggggggcgccgggtccgcaagggccacggggcgacaaaggggagactggcgagaggggggctgccggcatcaagggccaccgcggcctagaaaagagagacggcaatcctggttctgacggattgcctggtcgagatggttctcctggtggaaagggggatagaggggagaatggatctcctggcgccccaggtgcgccggggcatccaggcccgcccgggccggttggaccagcgggtaaatcgggcgacaggggggaaagcggtcctgcaggaccagcgggcgcaccggggcctgctgggagtagaggcgctccaggtccgcaaggtccccgaggggacaagggcgaaactggggagcgtggtgcggccggcataaagggacaccgaggactcgaaaaacgcgatggaaatcccggctccgacggactccctgggcgggatggcagtcccggaggtaagggagacagaggcgagaatggaagtcctggggcgcctggcgctccgggacatccagggccacccggaccggtaggaccggcaggaaaatccggtgaccgcggcgagtcaggtcccgcaggaccagcgggtgcacctgggccggcgggtagtcgtggggctcccgggccgcagggtccgagaggtgataagggagagacaggagaacgcggtgccgccggcattaaagggcaccgaggcctggagaaacgataa

SEQ ID NO: 77 - DNA, 1563 bp, synthetic construct
  source 1..1563: mol_type = other DNA; note = DNA sequence encoding 3A5D15E-5
gaagccgatggtaacccaggaagtgatggcctcccggggcgcgacggttctcctggcggaaaaggcgatcgtggagaaaatgggtcgccaggtgccccgggagcgcccgggcatcctggtccaccaggcccggttggtcctgcagggaagagtggggaccgcggagagtcgggtccagcgggacctgcaggcgctcctggcccagccggcagtcgcggtgcccctgggccacagggtcccagaggagacaagggggaaaccggggaaagaggagctgctggaataaagggacaccgggggctagagaaaagggaggccgacgggaacccaggatcagacggtctgccgggtcgggatgggagccctggcggaaaaggggatagaggcgaaaacggtagtccgggggcgcctggagcacccggccacccaggtcctcctggaccagttggtccggcaggtaaatccggggatcgcggcgagagcggccccgctggacctgcgggggcgccaggcccggcgggatcgcgaggtgcccctggtccgcaggggccgcgtggcgataagggtgagacaggtgagcggggagccgcgggcatcaaaggtcataggggcttagagaagcgtgaagcagatggaaatcccggatctgatggactgccgggacgagatggctcccctgggggcaaaggcgacagaggagaaaatggttcaccgggcgcaccaggtgctccaggccatccaggtccccccggcccagttggtcctgctggcaaaagtggagacagaggtgagtcgggacccgctgggcctgcgggagcaccaggtccggccggctcgcgcggtgctccaggcccccagggtccgcggggcgataagggcgagacaggagagcggggagccgcaggtattaaagggcatcgaggtttggagaaacgtgaagcagacggaaacccgggttcagatggactaccaggccgtgacggcagcccggggggaaagggtgaccgaggtgaaaacggttctcctggagcccccggtgccccggggcatcctgggcctccaggccccgtaggacccgcaggcaaatctggggaccgaggggaaagcggccccgctggtcctgcgggcgcccccggtcccgcgggttctcgtggtgcacctggcccccaaggtcctaggggtgacaagggggaaacgggggagcgtggggcagctgggataaaaggccaccggggtcttgaaaaacgcgaggcggatgggaatccgggaagcgacggcttaccgggacgggacggctcacccggggggaagggtgatcgcggggagaatggttcccccggtgctcctggggctcctgggcaccctggtccgcctggtcccgtcggaccggcagggaaatcaggggacagaggggaatccggacctgctggtcctgccggggctcccggtcctgctggttctcgtggagcccctggtcctcaagggccaaggggtgataagggtgaaactggcgagaggggagctgcagggatcaagggccaccgaggactcgaaaagaggtaa

SEQ ID NO: 78 - DNA, 1713 bp, synthetic construct
  source 1..1713: mol_type = other DNA; note = DNA sequence encoding 3A5D15R-6
gacggaaatcccggaagcgacggtcttcccggaagggatggctcccctggcgggaaaggtgatcgcggcgaaaacgggtctcccggcgcgcccggcgccccgggccaccctgggccacctggtccggttggtcctgctggcaaatcaggtgaccgtggggaatcggggccagctggtcctgctggggcgccaggacccgcaggcagtcgtggcgcgcccgggcctcaagggccacgaggtgataagggagagaccggcgagaggggggcggctggaatcaaacgggacggtaatcccggttcagacggcctcccgggacgcgacggctccccggggggtaaaggggatcgcggtgaaaacggatcgccaggtgcgccaggggcgcccggacaccctggtcctccggggcctgtcggcccggcaggcaagtctggcgacaggggcgagtctggtcctgcaggccccgcaggtgctcctggcccagcaggatcacgtggcgcccccggaccacaggggccgagaggggataagggcgaaactggtgaacggggggcggctggaattaagagagatggtaatcccggtagtgatgggctaccgggacgagacggttcacccgggggtaagggagatcgaggtgagaatggcagtccaggcgcccctggtgctcctgggcatcccggcccacccggtccggttggacccgcgggcaaatccggggaccggggggagagtggcccggccggtcctgcgggtgccccgggaccagcgggaagtaggggggctccggggccacaaggtcctcgtggagataagggcgaaacaggtgagagaggagctgcagggattaagagggacggaaatcccgggtcggatgggttgcctggacgggatggtagccccggtggtaaaggagaccgaggcgaaaacggatctcccggtgcgcctggagccccaggtcacccggggccacctggtcctgtaggccctgcaggtaagtcgggtgaccgcggagagagcggaccggccggtcctgcaggagcccctggacctgccggttcccggggagcaccaggcccccaaggaccgagaggtgacaagggggagacaggtgagcgtggggctgctgggataaaaagagatggtaacccgggctctgatgggctgcctggaagggatgggagcccaggtggaaaaggagatcggggtgagaacggttctcctggagccccgggagcccccggccatccggggccgccgggacctgtcggtcctgctggaaaatcaggcgatcgtggggaatcaggaccagctgggcctgctggagcaccggggccagcagggagcagaggtgctcctggacctcagggaccgcgaggcgacaaaggggagacgggcgaacgcggtgcggcaggtataaaacgagacgggaacccaggctctgatggtttaccaggtcgtgacggctcgcctggaggcaagggagatcgcggtgaaaatggttcccccggtgctcctggagcgcctgggcatccggggcctccaggtccggtaggtccagcaggcaagagcggggacaggggagaatccggaccagctggtcctgccggagcgccaggccccgcaggaagtcgaggggctcctggtccccaaggtcctcgtggcgacaaaggcgagaccggtgaacgcggcgctgcaggcatcaagagataa

SEQ ID NO: 79 - DNA, 1749 bp, synthetic construct
  source 1..1749: mol_type = other DNA; note = DNA sequence encoding 3A5D15KR-6
gacggtaaccctggaagtgacggattgccggggcgagacggttcacccggaggaaagggcgatcgcggcgaaaatgggtcaccgggcgctcctggggcaccagggcatccgggtccccccggtcctgttgggccggcgggtaagtctggtgatcgaggcgagtctggccctgcgggtcctgctggtgcacctggacctgccggatcgagaggggctccagggccgcaaggacctaggggtgacaaaggcgaaacgggtgagcgaggagccgccggaattaaggggaaaagggatggcaaccccgggtccgatggcctgccaggacgcgatgggtcgcccggaggcaagggtgacagaggggagaatggctctccaggtgcaccaggtgccccggggcaccccggtccgcctggaccagttggaccggcgggaaagtctggagatcgcggggagagtggaccggctggtcctgcaggggcaccgggtcccgctgggtctcgcggagcgcctggcccccaaggacccagaggggataagggcgaaactggagagcgtggcgcggcaggaataaagggcaaacgtgatggcaatccagggtcggacggacttcctggccgggacggttccccagggggaaagggtgacagaggcgaaaacggctcgcccggtgcgccaggggcgcctggtcatccggggcctccgggtccagtgggaccagccggaaaaagcggggatcggggggaatctggaccggctggaccagccggcgcaccaggccccgccggatcgaggggggcgcccggaccgcagggtcctagaggggataaaggtgagaccggcgagaggggcgcagctgggataaagggtaagcgggacggtaaccccggctccgacggtctcccaggacgagacgggtcaccgggtggtaagggagaccgaggcgaaaatgggtcacctggtgcacccggcgcccctggacaccccggtcctcctggaccagtgggacccgcagggaagagcggtgacagaggggagagtgggcctgcaggaccagctggcgctccgggaccggccggaagtcggggtgctcccggcccccaagggcctagaggggataaaggtgagaccggggaacgtggcgcggccggtatcaagggcaaacgcgacggcaacccaggttcggatggactaccagggcgagatggttcacctggcggtaaaggcgatcggggggaaaatggcagccccggtgctcctggagcaccgggtcatcctggtccgcctggtcctgttggaccggctgggaaatccggtgaccgcggagaatccggcccggccggtccggctggagcccctgggccggctggcagtcgtggcgcgcctggcccacagggtccgcgtggagataaaggggaaacaggtgagaggggcgcagcgggaatcaaggggaaacgggatggcaacccggggagcgacgggttacccgggcgagacggttccccaggaggcaagggcgatcgtggcgagaatggtagccccggtgctccaggagcacctggccacccagggccaccaggaccggtaggacccgctggtaaatcaggcgatcggggtgagagtggccctgcgggacccgcgggcgcccccggacctgccgggagccgcggtgctcctggaccacaaggtcctaggggcgacaaaggtgaaacaggggaacgtggcgctgcggggattaaaggaaaaaggtaa

SEQ ID NO: 80 - DNA, 1731 bp, synthetic construct
  source 1..1731: mol_type = other DNA; note = DNA sequence encoding 3A5D15EKR-6
gacggaaaccctggctcggatggtcttccaggacgggatggcagtcccggcggaaaaggcgaccggggagaaaacggttcacccggtgctcctggagcaccaggacatcctgggccacccggccccgttggtccggcggggaaatcaggcgacaggggcgaaagtgggcctgccgggcctgcgggagccccgggtccggcaggtagccgaggggcaccaggccctcaagggccacgaggtgacaagggagaaacaggcgaaaggggtgctgctggaatcgagaaacgtgatgggaatcccgggtcagacggcctaccgggacgggatgggtcccccggcggcaaaggggaccgaggggagaatggttcgcctggtgccccaggcgcgccgggtcatcctggtcccccgggacccgtcggtcctgctggcaaaagtggggatcgtggagaaagtggacctgccggacctgccggggctcctggtcctgctggatcgcgcggcgcaccaggacctcaaggtcctagaggagacaaaggggagacgggagaaagaggagctgcagggatagaaaaacgggatgggaatcctggaagcgatgggttaccaggcagggacggaagccccggcgggaagggggacaggggggagaatggttcaccaggtgcgcccggagccccgggacatcccgggccgcctggtccggtagggcctgcaggtaaatccggtgatagaggagaatccggacctgcggggccagccggagcgccggggccggcgggtagcaggggcgcaccgggacctcaagggccacggggtgataagggagaaaccggtgagaggggcgcggctggaattgagaagcgtgatggtaaccctgggtccgatggactgcccggccgagacggctcgcctggcggcaagggcgaccgcggcgagaatgggtctcccggtgctcctggtgctcctggacaccctggtcctcccggtccggtgggtcctgccggcaagagtggggacagaggggaatcggggccggctggaccggcgggtgcaccgggtcccgctggctcacgaggtgcgccggggccacaaggcccacgcggcgataagggggagactggtgagcgtggagctgcaggaatcgagaagcgcgatggcaacccaggtagcgacggattgccaggtcgtgacggatctcctgggggtaagggtgatcgaggagaaaatggctcaccgggtgctcctggggcgcccggccacccgggacctcctggtcctgtaggtcccgccggcaaatcgggcgaccggggtgagtctgggcctgcaggcccggccggtgccccaggtccagcagggtctcgtggcgcgcccggtccccagggtcctcgtggggataagggcgagacgggagaaagaggtgcggcaggcatagaaaagcgcgatgggaaccctggatctgatgggctcccagggagagacggaagccccggcggaaaaggtgatcggggcgaaaacggaagtccaggtgcgcccggagcacccggccacccaggtccacccggaccggttggtcccgctgggaaatctggtgacagaggggagtccgggccagcagggccggccggcgcaccaggaccagctggttctcgtggtgcccctggacctcaaggtcctaggggggacaaaggcgagaccggggaacgcggtgcggctgggattgagaagcgctaa

SEQ ID NO: 81 - DNA, 1731 bp, synthetic construct
  source 1..1731: mol_type = other DNA; note = DNA sequence encoding 3A5D15G-6
gacggcaatcctggatctgacgggctgcctggccgtgacgggagcccagggggtaaaggcgaccgcggagaaaatggtagccctggcgctcctggtgctcccggtcatcctggtcccccgggaccagtggggccggctggaaaaagcggtgaccgtggtgaatctggcccagcgggacctgcgggagcccctggtcctgccggttctcgtggcgcacccggacctcaaggtccgcggggtgataaaggcgagacaggggagcgaggtgccgcaggcattggaaaaagggacggcaatccgggttcagacggcttgccaggaagggatggctcgccgggtggtaagggagacaggggagaaaacggttccccaggtgctcctggcgcacctggccaccctggtcctccggggcctgtaggaccagctggcaagagtggagatcgcggagagtctgggcctgcgggtccggcaggtgctcccggacccgccggatcacgcggtgctcctggaccgcaaggtccgcggggtgacaagggagagactggggagaggggtgcggcgggtattggtaagcgtgatggcaatccaggcagcgacggtctaccggggcgggatgggagtcccggtgggaagggggataggggtgagaacggctctccaggggctcccggtgcccctgggcatcctggtcctcctgggcctgtgggtcctgccggcaagtcaggggatcgaggcgagagtggtcctgctggtcctgctggggcgccaggaccagcggggtctcgaggcgcccctggcccgcagggtccaagaggtgataagggggagaccggggaacgaggagccgctgggatagggaagcgcgacggaaatcccgggagtgatgggcttccaggccgtgatggaagtcccggagggaagggagatcggggcgaaaacggttctcccggtgctcctggagcgcccggacaccccggcccaccaggccctgttgggccggccgggaaaagcggcgatcgtggcgaatctggtcctgcgggtccagctggtgctcctgggccggcaggttctcgtggtgcacccggaccgcagggacccagaggagataaaggggaaacgggtgagcgaggggcagcaggtatcgggaaaagggacggtaaccctggctccgatggcttaccggggcgagacggatcgccggggggtaaaggagaccggggagagaacggttcaccaggcgcacccggcgctccagggcatcctgggccacccggcccagttggtcctgctggtaaatcgggggaccgaggcgaatcaggacctgcaggccctgcgggtgcccccggccccgctgggagtcgtggtgcacctgggccacaaggcccgcgcggcgacaagggggagacgggagagcgcggtgccgctggaatcggcaagagagatggtaaccccgggagcgacggactcccaggcagagatgggtccccgggcggcaaaggagacagaggtgaaaatggatcacctggtgcgcctggtgctcctggacacccaggaccgccaggtccagtcggtcctgccgggaaatcgggtgatcgtggtgaatccgggcctgcaggtcccgctggagcgccgggtcccgcagggtcgaggggcgcgccaggtccacaaggtcctcggggcgataagggcgaaacaggtgaaagaggcgcggccggcataggaaaaagataa